European Patent Specification EP 3 607 044 B1, published November 13, 2024. Title: CLEANING COMPOSITIONS AND USES THEREOF. Applicant: Novozymes A/S. The sequence listing filed with the application follows.

SEQUENCE LISTING (104 sequences)

SEQ ID NO: 1 - protein, 182 aa, Bacillus sp-62451
LPPDLPSKSTTQAQLNSLNVKNEESMSGYSREKFPHWISQGDGCDTRQVILKRDADNYSGNCPVTSGKWYSYYDGITFNDPSQLDIDHVVPLAEAWRSGASSWSTAKREDFANDLNGPQLIAVSASSNRSKGDQDPSTWQPPRAGANCAYAKMWINTKYNWGLHLQSSEKTALQGMLNSCSY

SEQ ID NO: 2 - protein, 182 aa, Bacillus horikoshii
LPPGTPTKSEAQNQLNSLTVKSEGSMTGYSRDLFPHWSGQGNGCDTRQIVLQRDADYYTGTCPTTSGKWYSYFDGVIVYSPSEIDIDHIVPLAEAWRSGASSWTTEQRRAFANDLNGPQLIAVTASVNRSKGDQDPSTWQPPRAGARCAYAKWWINTKHRWNLHLQSSEKSSLQTMLNGCAY

SEQ ID NO: 3 - protein, 182 aa, Bacillus sp-62520
LPPGTPSKSEAQSQLNALTVKPEDPMTGYSRDHFPHWISQGNGCNTRQIVLQRDADYYSGACPVTTGKWYSYFDGVIVYSPSEIDIDHIVPLAEAWRSGASSWTTEKRRSFANDLNGPQLIAVTASVNRSKGDQDPSTWQPPRAGARCAYAKWWINTKHRWGLHLQSSEKSSLQSMLNGCAY

SEQ ID NO: 4 - protein, 182 aa, Bacillus sp-62520
LPPGTPSKSEAQSQLNALTVKPEDPMTGYSRDHFPHWISQGNGCNTRQIVLQRDADYYSGACPVTTGKWYSYFDGVIVYSPSEIDIDHIVPLAEAWRSGASSWTTEQRRSFANDLNGPQLIAVTASVNRSKGDQDPSTWQPPRAGARCAYAKWWINTKHRWGLHLQSSEKSSLQSMLNGCAY

SEQ ID NO: 5 - protein, 182 aa, Bacillus horikoshii
LPPGTPSKSEAQSQLNSLTVKSEDPMTGYSRDHFPHWSGQGNGCDTRQIVLQRDADYYSGNCPVTSGKWYSYFDGVIVYSPSEIDIDHVVPLAEAWRSGASSWTTEQRRSFANDLNGPQLIAVTASVNRSKGDQDPSTWQPPRAGARCAYAKWWINTKHRWNLHLQSSEKSALQTMLNGCVY

SEQ ID NO: 6 - protein, 182 aa, Bacillus horikoshii
LPPGTPSKSEAQSQLNSLTVKTEDPMTGYSRDLFPHWSGQGSGCDTRQIVLQRDADYFTGTCPTTSGKWYSYFDGVIVYSPSEIDVDHIVPLAEAWRSGASSWTTEQRRAFANDLTGPQLIAVTASVNRSKGDQDPSTWQPPRAGARCAYAKWWINTKHRWNLHLQSSEKSSLQTMLNGCAY

SEQ ID NO: 7 - protein, 182 aa, Bacillus sp-16840
LPPGTPSKSEAQSQLNALTVKAEDPMTGYSRNLFPHWNSQGNGCNTRQLVLQRDADYYSGNCPVTSGRWYSYFDGVVVTSPSEIDIDHIVPLAEAWRSGASSWTTEKRKEFANDLNGPQLIAVTASVNRSKGDQDPSTWQPPRAAARCGYAKWWINTKYRWDLSLQSSEKSSLQTMLNTCSY

SEQ ID NO: 8 - protein, 182 aa, Bacillus sp-16840
LPPGTPSKSQAQSQLNALTVKAEDPMTGYSRNLFPHWSSQGNGCNTRQLVLQRDADYYSGNCPVTSGRWYSYFDGVVVTSPSEIDIDHIVPLAEAWRSGASSWTTEKRREFANDLNGPQLIAVTASVNRSKGDQDPSTWQPPRVAARCGYAKWWINTKYRWDLSLQSSEKSSLQTMLNTCSY

SEQ ID NO: 9 - protein, 182 aa, Bacillus sp-62668
LPPGTPSKSEAQSQLTSLTVKPEDPMTGYSRDHFPHWISQGNGCNTRQIVLQRDADYYSGNCPVTTGKWYSYFDGVIVYSPSEIDIDHIVPLAEAWRSGASSWTAEQRRNFANDLNGPQLIAVTASVNRSKGDQDPSTWQPPRTGARCAYAKWWINTKYRWGLHLQSSEKSSLQSMLNGCAY

SEQ ID NO: 10 - protein, 183 aa, Bacillus sp-13395
AFPPGTPSKSTAQSQLNSLTVKSEGSMTGYSRDKFPHWISQGDGCDTRQLVLKRDGDYYSGNCPVTSGKWYSYYDGIAVYSPSEIDIDHIVPLAEAWRSGASGWTTEKRQNFANDLNGPQLIAVTASVNRSKGDQDPSTWQPPRSGSHCAYAKMWVNTKYRWGLHLQSAEKSALQSMLNACSY

SEQ ID NO: 11 - protein, 185 aa, Bacillus horneckiae
ASAFPPGTPSKSTAQSQLNSLTVKSEGSMTGYSRDKFPHWISQGDGCDTRQLVLKRDGDYYSGNCPVTSGKWYSYYDGITVYSPSEIDIDHIVPLAEAWRSGASGWTTEKRQSFANDLNGPQLIAVTASVNRSKGDQDPSTWQPPRSGSHCAYAKMWVNTKYRWGLHVQSAEKSALQSMLNACSY

SEQ ID NO: 12 - protein, 182 aa, Bacillus sp-11238
FPPEIPSKSTAQSQLNSLTVKSEDAMTGYSRDKFPHWISQGDGCDTRQMVLKRDADYYSGSCPVTSGKWYSYYDGITVYSPSEIDIDHIVPLAEAWRSGASSWTTEKRRNFANDLNGPQLIAVTASVNRSKGDQDPSTWQPPRSGARCAYAKMWVNTKYRWGLHLQSAEKSGLESMLNTCSY

SEQ ID NO: 13 - protein, 182 aa, Bacillus cibi [sequence omitted]

SEQ ID NO: 14 - protein, 182 aa, Bacillus sp-18318
FPPGTPSKSTAQSQLNSLTVKSEGSMTGYSRDKFPHWIGQGSGCDTRQLVLQRDADYYSGSCPVTSGKWYSYYDGVTFYDPSDLDIDHVVPLAEAWRSGASSWSTQKRKDFANDLSGPQLIAVSASSNRSKGDQDPSTWQPTRSGAACGYSKWWISTKHKWGLSLQSSEKNALQGMLNSCVY

SEQ ID NO: 15 - protein, 182 aa, Bacillus idriensis
LPPGTPSKSTAQSQLNALTVQTEGSMTGYSRDKFPHWISQGNGCDTRQVVLQRDADYYSGTCPVTSGKWYSYYDGVTLYNPSDLDIDHVVALAEAWRSGASSWTTDKREDFANDLSGTQLIAVSASTNRSKGDQDPSTWQPPRSGAACGYAKWWISTKYKWNLNLQSSEKTALQSMLNSCSY

SEQ ID NO: 16 - protein, 182 aa, Bacillus algicola
FPPGTPSKSEAQSQLNSLTVQSEGSMSGYSRDKFPHWIGQGNGCDTRQLVLQRDADYYSGDCPVTSGKWYSYFDGVTVYDPSDLDIDHMVPMAEAWRSGASSWSTQKREDFANDLSGPHLIAVTASSNRSKGDQDPSTWKPTRYGAHCGYAKWWINTKYVYDLTLQSSEKTELQSMLNTCSY

SEQ ID NO: 17 - protein, 182 aa, Enviromental sample J
LPPNIPSKADALTKLNALTVQTEGPMTGYSRDLFPHWSSQGNGCNTRHVVLKRDADSVVDTCPVTTGRWYSYYDGLVFTSASDIDIDHVVPLAEAWRSGASSWTSTKRQSFANDLNGPQLIAVSATSNRSKGDQDPSTWQPPRAGARCAYAKMWVETKSRWGLTLQSSEKAALQTAINACSY

SEQ ID NO: 18 - protein, 182 aa, Bacillus vietnamensis
FPPGTPSKSTAQSQLNALTVKSESSMTGYSRDKFPHWIGQRNGCDTRQLVLQRDADSYSGSCPVTSGSWYSYYDGVTFTDPSDLDIDHVVPLAEAWRSGASSWTTAKREDFANDLSGPQLIAVSASSNRSKGDQDPSTWQPPRSGAACGYSKWWISTKYKWGLSLQSSEKTALQGMLNSCIY

SEQ ID NO: 19 - protein, 182 aa, Bacillus hwajinpoensis
IPPGTPSKSAAQSQLDSLAVQSEGSMSGYSRDKFPHWIGQGNGCDTRQLVLQRDADYYSGDCPVTSGKWYSYFDGVQVYDPSYLDIDHMVPLAEAWRSGASSWSTQKREDFANDLDGPHLIAVTASSNRSKGDQDPSTWKPTRYSAHCGYAKWWINTKYVYDLNLQSSEKSALQSMLNTCSY

SEQ ID NO: 20 - protein, 182 aa, Paenibacillus mucilaginosus
LPPGTPSKSTAQSQLNSLTVKSESTMTGYSRDKFPHWTSQGGGCDTRQVVLKRDADYYSGSCPVTSGKWYSYYDGITVYSPSEIDIDHIVPLAEAWRSGASSWTTEKRQNFANDLGGPQLIAVTASSNRAKGDQDPSTWKPTRSGAHCAYAKWWINTKYRWGLHLQSSEKTALQSMLNTCSY

SEQ ID NO: 21 - protein, 182 aa, Bacillus indicus
TPPGTPSKSTAQTQLNALTVKTEGSMTGYSRDLFPHWISQGSGCDTRQVVLKRDADYYSGSCPVTSGKWYSYYDGVTFYDPSDLDIDHIVPLAEAWRSGASSWTTSKRQDFANDLSGPQLIAVSASTNRSKGDQDPSTWQPPRAGAACGYSKWWISTKYKWGLSLQSSEKTALQGMLNSCSY

SEQ ID NO: 22 - protein, 182 aa, Bacillus marisflavi
TPPVTPSKATSQSQLNGLTVKTEGAMTGYSRDKFPHWSSQGGGCDTRQVVLKRDADSYSGNCPVTSGSWYSYYDGVKFTNPSDLDIDHIVPLAEAWRSGASSWTTAQREAFANDLSGSQLIAVSASSNRSKGDQDPSTWQPPRAGAKCGYAKWWISTKSKWNLSLQSSEKTALQGMLNSCVY

SEQ ID NO: 23 - protein, 184 aa, Bacillus luciferensis
ASLPPGIPSLSTAQSQLNSLTVKSEGSLTGYSRDVFPHWISQGSGCDTRQVVLKRDADYYSGNCPVTSGKWYSYYDGVTVYSPSEIDIDHVVPLAEAWRSGASSWTTEKRQNFANDLNGPQLIAVTASSNRSKGDQDPSTWQPTRTGARCAYAKMWINTKYRWGLHLQSSEKSALQSMLNTCSY

SEQ ID NO: 24 - protein, 182 aa, Bacillus marisflavi
TPPVTPSKETSQSQLNGLTVKTEGAMTGYSRDKFPHWSSQGGGCDTRQVVLKRDADSYSGNCPVTSGSWYSYYDGVKFTHPSDLDIDHIVPLAEAWRSGASSWTTAQREAFANDLSGSQLIAVSASSNRSKGDQDPSTWQPPRAGAKCGYAKWWISTKSKWNLSLQSSEKTALQGMLNSCVY

SEQ ID NO: 25 - protein, 182 aa, Bacillus sp. SA2-6
LPSGIPSKSTAQSQLNSLTVKSEGSMTGYSRDKFPHWISQGGGCDTRQVVLKRDADYYSGNCPVTSGKWYSYYDGISVYSPSEIDIDHVVPLAEAWRSGASSWTTTKRQNFANDLNGPQLIAVTASVNRSKGDQDPSTWQPPRYGARCAYAKMWINTKYRWDLNLQSSEKSSLQSMLDTCSY

SEQ ID NO: 26 - protein, 191 aa, Pyrenochaetopsis sp.
LPSPLLIARSPPNIPSATTAKTQLAGLTVAPQGPQTGYSRDLFPHWITQSGTCNTREVVLKRDGTNVVTNSACASTSGSWLSPYDGKTWDSASDIQIDHLVPLSNAWKSGAAAWTTAQRQAFANDLTHPQLVAVTGSVNESKGDDGPEDWKPPLASYYCTYASMWTAVKSNYKLTITSAEKSALTSMLATC

SEQ ID NO: 27 - protein, 190 aa, Vibrissea flavovirens
TPLPIIARTPPNIPTTATAKSQLAALTVAAAGPQTGYSRDLFPTWITISGTCNTRETVLKRDGTNVVVDSACVATSGSWYSPYDGATWTAASDVDIDHMVPLSNAWKSGASAWTTAQRQTFANDLTNPQLLAVTDNVNQAKGDSGPEDWKPSLTSYWCTYAKMWVKVKTVYDLTITSAEKTALTTMLNTC

SEQ ID NO: 28 - protein, 192 aa, Setosphaeria rostrata
APTSSPLVARAPPNVPSKAEATSQLAGLTVAPQGPQTGYSRDLFPHWITQSGTCNTRETVLKRDGTNVVTNSACASTSGSWFSPYDGATWTAASDVDIDHMVPLSNAWKSGAASWTTARRQAFANDLTNPQLLAVTDNVNQAKGDKGPEDWKPPLTSYYCTYSKMWIKVKSVWGLTITSAEKSALTSMLATC

SEQ ID NO: 29 - protein, 192 aa, Endophragmiella valdina
APVPGHLMPRAPPNVPTTAAAKTALAGLTVQAQGSQTGYSRDLFPHWITQSGTCNTREVVLKRDGTNVVTDSACAATSGTWVSPYDGATWTAASDVDIDHMVPLSNAWKSGAASWTTAQRQAFANDLTNPQLLAVTDNVNQSKGDKGPEDWKPPLTSYYCTYAKMWVKVKSVYSLTITSAEKTALTSMLNTC

SEQ ID NO: 30 - protein, 190 aa, Corynespora cassiicola
LPAPLVPRAPPGIPTTSAARSQLAGLTVAAQGPQTGYSRDLFPHWITQSGSCNTREVVLARDGTGVVQDSSCAATSGTWRSPFDGATWTAASDVDIDHMVPLSNAWKSGAASWTTSRRQAFANDLTNPQLIAVTDNVNQSKGDKGPEDWKPPLTSYYCTYAKMWVRVKSVYSLTITSAEKSALTSMLDTC

SEQ ID NO: 31 - protein, 192 aa, Paraphoma sp. XZ1965
APAPVHLVARAPPNVPTAAQAQTQLAGLTVAAQGPQTGYSRDLFPHWITQSGACNTRETVLKRDGTGVVQDSACAATSGTWKSPYDGATWTAASDVDIDHMVPLSNAWKSGAASWTTARRQAFANDLTNPQLLAVTDNVNQAKGDKGPEDWKPPLTSYYCIYARMWIKVKSVYSLTITSAEKSALTSMLGTC

SEQ ID NO: 32 - protein, 186 aa, Monilinia fructicola
TPVPAPTGIPSTSVANTQLAALTVAAAGSQDGYSRDLFPHWITISGACNTRETVLKRDGTNVVVNSACAATSGTWVSPYDGATWTAASDVDIDHLVPLSNAWKAGASSWTTAQRQAFANDLVNPQLLAVTDSVNQGKSDSGPEAWKPSLKSYWCTYAKMWIKVKYVYDLTITSAEKSALVTMMDTC

SEQ ID NO: 33 - protein, 190 aa, Curvularia lunata
APAPLSARAPPNIPSKADATSQLAGLTVAAQGPQTGYSRDLFPHWITQSGTCNTRETVLKRDGTNVVTSSSCAATSGTWFSPYDGATWTAASDVDIDHVVPLSNAWKSGAASWTTARRQAFANDLTNPQLIAVTDSVNQAKGDKGPEDWKPPLSSYYCTYSKMWIKVKSVYGLTVTSAEKSALSSMLATC

SEQ ID NO: 34 - protein, 191 aa, Penicillium reticulisporum
LPAPEALPAPPGVPSASTAQSELAALTVAAQGSQDGYSRSKFPHWITQSGSCDTRDVVLKRDGTNVVQSASGCTITSGKWVSPYDGATWTASSDVDIDHLVPLSNAWKSGASGWTTAARQAFANDLTNPQLLVVTDNVNESKGDKGPEEWKPPLTSYYCTYAEMWVKVKSVYKLTITSAEKSALTSMLSTC

SEQ ID NO: 35 - protein, 191 aa, Penicillium quercetorum
LPAPEPAPSPPGIPSASTARSELASLTVAPQGSQDGYSRAKFPHWIKQSGSCDTRDVVLERDGTNVVQSSTGCTITGGTWVSPYDGATWTASSDVDIDHLVPLSNAWKSGASAWTTAQRQAFANDLTNPQLVAVTDNVNEAKGDKGPEEWKPPLTSYYCTYAEMWVKVKSVYKLTITSAEKSALSSMLNTC

SEQ ID NO: 36 - protein, 192 aa, Setophaeosphaeria sp.
LPAPVTLEARAPPNIPSTASANTLLAGLTVAAQGSQTGYSRDLFPHWITQSGTCNTRETVLKRDGTGVVTDSACASTSGSWYSVYDGATWTAASDVDIDHVVPLSNAWKSGAASWTTARRQSFANDLTNPQLIAVTDNVNQAKGDKGPEDWKPPLTSYYCTYAKMWVKVKSVYSLTITSAEKTALTSMLNTC

SEQ ID NO: 37 - protein, 192 aa, Alternaria sp. XZ2545
LPAPVTLEARAPPNIPTTAAAKTQLAGLTVAAQGPQTGYSRDLFPHWITQSGTCNTRETVLKRDGTGVVTDSACASTSGSWFSVYDGATWTAASDVDIDHVVPLSNAWKSGAASWTTARRQSFANDLTNPQLIAVTDNVNQAKGDKGPEDWKPPLTSYYCTYAKMWVKVKSVYALTITSAEKTALTSMLNTC

SEQ ID NO: 38 - protein, 192 aa, Alternaria sp.
LPAPVTLEARAPPNIPTTAAAKTQLAGLTVAAQGPQTGYSRDLFPHWITQSGSCNTREVVLQRDGTGVVTDSACAATSGSWYSVYDGATWTAASDVDIDHMVPLSNAWKSGAASWTTARRQAFANDLTNPQLLAVTDNVNQAKGDKGPEDWKPPLTSYYCTYAKMWVKVKSVYALTITSAEKTALTSMLNTC

SEQ ID NO: 39 - protein, 186 aa, Trichoderma reesei
APLPAPPGIPSEDTARTQLAGLTVAVVGSGTGYSRDLFPTWDAISGNCNAREYVLKRDGEGVQVNNACEAQSGSWISPYDNASFTNASSLDIDHMVPLKNAWISGASTWTTAQREALANDVSRPQLWAVSASSNRSKGDRSPDQWKPPLTSFYCTYAKSWIDVKSYYKLTITSAEKTALSSMLDTC

SEQ ID NO: 40 - protein, 188 aa, Chaetomium thermophilum
APAPQPTPPGIPSRSTAQSYLNSLTVAASYDDGNYNRDLFPHWNTVSGTCNTREYVLKRDGSNVVTNSACQATSGTWYSPYDGATWTAASDIDIDHMVPLKNAWISGANTWSSSKRSSFANDINSPQLWAVTDSVNQSKGDKSPDKWKPPLTTFYCTYAKSWITVKYNYNLTITSAEKSALQNMINTC

SEQ ID NO: 41 - protein, 190 aa, Scytalidium thermophilum
LPAPAPMPTPPGIPSKSTAQSQLNALTVKASYDDGKYKRDLFPHWNTVSGTCNTREYVLKRDGVNVVTNSACAATSGTWYSPFDGATWTAASDVDIDHMVPLKNAWISGANNWTSTKRTQFANDINLPQLWAVTDDVNQAKGDKSPDKWKPPLTSFYCTYAKSWITVKYNYGLSITSAEKSALTSMINTC

SEQ ID NO: 42 - protein, 186 aa, Metapochonia suchlasporia
VPVPAPPGIPSTSTAKTLLAGLKVAVPLSGDGYSREKFPLWETIQGTCNAREFVLKRDGTDVKTNNACVAESGNWVSPYDGVKFTAARDLDIDHMVPLKNAWISGASQWTTERRKALANDITRPQLWAVSAHANRGKSDDSPDEWKPPLKTFWCTYAKSWVQVKSFYELTITDAEKGALAGMLDSC

SEQ ID NO: 43 - protein, 198 aa, Daldinia fissa
APAPIPVAEPAPMPMPTPPGIPSASSAKSQLASLTVKAAVDDGGYQRDLFPTWDTITGTCNTREYVLKRDGANVQVGSDCYPTSGTWTSPYDGGKWTSPSDVDIDHMVPLKNAWVSGANKWTTAKREQFANDVDRPQLWAVTDNVNSSKGDKSPDTWKPPLTSFYCTYASAYVAVKSYWGLTITSAEKSALSDMLGTC

SEQ ID NO: 44 - protein, 188 aa, Acremonium sp. XZ2007
LPLQSRDPPGIPSTATAKSLLNGLTVKAWSNEGTYDRDLFPHWQTIEGTCNAREYVLKRDGQNVVVNSACTAQSGTWKSVYDGETTNSASDLDIDHMIPLKNAWISGAATWTTAQRTSFANDISSPQLWAVTAGVNRSKSDRSPDTWVPPLASFHCTYGKAWVQVKSKWALSITSAEKSALTGLLNKC

SEQ ID NO: 45 - protein, 182 aa, Acremonium dichromosporum
IPPGIPSEATARSLLSSLTVAPTVDDGTYDRDLFPHWSSVEGNCNAREFVLRRDGDGVSVGNDCYPTAGTWTCPYDGKRHSVPSDVSIDHMVPLHNAWMTGASEWTTAEREAFANDIDGPQLWAVTSTTNSQKGSDAPDEWQPPQTSIHCKYAAAWIQVKSTYDLTVSSAEQAALEEMLGRC

SEQ ID NO: 46 - protein, 188 aa, Sarocladium sp. XZ2014
VPIPLPDPPGIPSSSTANTLLAGLTVRASSNEDTYNRDLFPHWVAISGNCNAREYVLRRDGTNVVVNTACVPQSGTWRSPYDGESTTNASDLDIDHMVPLKNAWISGAASWTTAKRQDFANDVSGPQLWAVTAGVNRSKGDKSPDSWVPPLASFHCTYARSWIQVKSSWALSVTSAEKAALTDLLSTC

SEQ ID NO: 47 - protein, 186 aa, Metarhizium sp. HNA15-2
VPVPAPPGIPTASTARTLLAGLKVATPLSGDGYSRTLFPTWETIEGTCNAREFVLKRDGTDVQTNTACVAQSGNWVSPYDGVAFTAASDLDIDHMVPLKNAWISGASQWTTDKRKGLANDITRPQLWAVSAHANRAKGDSSPDEWKPPLKTFWCTYARSWVQVKSYYALTITDAEKGALSGMLDSC

SEQ ID NO: 48 - protein, 188 aa, Acremonium sp. XZ2414
APIAVRDPPGIPSASTANTLLAGLTVRASSNEDSYDRNLFPHWSAISGNCNAREFVLERDGTNVVVNNACVAQSGTWRSPYDGETTGNASDLDIDHMVPLKNAWISGASSWSTTRRQEFANDVSGPQLWAVTAGVNRSKGDRSPDSWVPPLASFHCTYAKSWVQVKSSWSLSVTSAEKAALSDLLGTC

SEQ ID NO: 49 - protein, 186 aa, Isaria tenuipes
APVPEPPGIPSTSTAQSDLNSLQVAASGSGDGYSRAEFPHWVSVEGSCDSREYVLKRDGQDVQADSSCKITSGTWVSPYDATTWTNSSKVDIDHLVPLKNAWISGASSWTKAQRQDFANDIKRPQLYAVSENANRSKGDRSPDGWKPPLKSFYCTYAKSWVAVKSYYKLTITSAEKSALGDMLDTC

SEQ ID NO: 50 - protein, 184 aa, Scytalidium circinatum
APPGIPSASTASSLLGELAVAEPVDDGSYDRDLFPHWEPIPGETACSAREYVLRRDGTGVETGSDCYPTSGTWSSPYDGGSWTAPSDVDIDHMVPLKNAWISGASEWTTAEREAFANDIDGPQLWAVTDEVNQSKSDQSPDEWKPPLSSFYCTYACAWIQVKSTYSLSISSAEQAALEDMLGSC

SEQ ID NO: 51 - protein, 186 aa, Metarhizium lepidiotae
VPVPAPPGIPTASTARTLLAGLKVATPLSGDGYSRTLFPTWETIEGTCNAREFVLKRDGTDVQTNTACVAESGNWVSPYDGVSFTAASDLDIDHMVPLKNAWISGASQWTTDKRKDLANDITRPQLWAVSAHANRSKGDSSPDEWKPPLQTFWCTYSKSWIQVKSHYSLTITDAEKGALSGMLDSC

SEQ ID NO: 52 - protein, 226 aa, Thermobispora bispora
LDIADGRPAGGKAAEAATGTSPLANPDGTRPGLAAITSADERAEARALIERLRTKGRGPKTGYEREKFGYAWADSVDGIPFGRNGCDTRNDVLKRDGQRLQFRSGSDCVVISMTLFDPYTGKTIEWTKQNAAEVQIDHVVPLSYSWQMGASRWSDEKRRQLANDPLNLMPVDGATNSRKGDSGPASWLPPRREIRCAYVVRFAQVALKYDLPVTTADKETMLQQCS

SEQ ID NO: 53 - protein, 191 aa, Sporormia fimetaria
LPAPVLEKRTPPNIPSTSTAQSLLSGLTVAPQGSQTGYSRDLFPHWITVSGTCNTRETVLKRDGSNVVTDSACASVSGSWYSTYDGATWTAASDVDIDHVVPLSNAWKSGAASWTTARRQAFANDLTNPQLIAVTDNVNQAKGDQGPESWKPPLTSYYCTYAKMWVKVKSVYSLTVTSAEKSALSSMLGTC

SEQ ID NO: 54 - protein, 193 aa, Pycnidiophora cf.dispera
LPAPAPVLVAREPPNIPSTSSAQSMLSGLTVKAQGPQDGYSRDLFPHWITISGTCNTRETVLKRDGTNVVTNSACASTSGSWYSPYDGATWTAASDVDIDHIVPLSNAWKSGAASWTTSRRQQFANDLTNPQLIAVTDSVNQAKGDKGPEDWKPSRTSYHCTYAKMWIKVKSVYSLTVTSAEKSALTTMLNTC

SEQ ID NO: 55 - protein, 199 aa, Enviromental sample D
DTDPEPVAGSALEALAGLEVKGPGPDTGYERALFGPPWADVDGNGCDTRNDILARDLTDLTFSTRGDVCEVRTGTFDDPYTGETIDFRRGNATSAAVQIDHVVPLLDAWRKGARAWDDETRRQFANDPLNLLASDGPANQSKGARDASAWLPPNHAFRCPYVARQIAVKAAYELSVTPSESEAMARVLADCPAEPLPAG

SEQ ID NO: 56 - protein, 199 aa, Enviromental sample O
DDEPEPARGSALEALARLEVVGPGPDTGYERELFGPAWADVDGNGCDTRNDILARDLTDLTFSTRGEVCEVRTGTFQDPYTGETIDFRRGNATSMAVQIDHVVPLMDAWRKGARAWDDETRRQFANDPLNLLASDGPANQSKGARDASAWLPPNHAFRCPYVARQIAVKTAYELSVTPSESEAMARVLEDCPAEPVPAG

SEQ ID NO: 57 - protein, 186 aa, Clavicipitaceae sp-70249
VPVPAPPGIPSTSTAKTLLAGLKVATPLSGDGYSRDKFPTWETIQGTCNAREFVIKRDGTDVKTNSACVAESGNWVSPYDGVKFTAARDLDIDHMVPLKNAWISGASQWTTEQRKALANDITRPQLWAVSAHANRGKSDDSPDEWKPPLKTFWCTYAKSWVQVKSFYKLTITDTEKGALAGMLDTC

SEQ ID NO: 58 - protein, 187 aa, Westerdykella sp. AS85-2
FPAPASVLEARAPPNIPSASTAQSLLVGLTVQPQGPQDGYSRDLFPHWITISGTCNTRETVLKRDGSNVVTNSACAATSGTWYSPYDGATWTSASDVDIDHLVPLSNAWKSGAASWTTAKRQQFANDLTNPQLLAVTDRVNQAKGDKGPEAWKPSLASYHCTYAKMWVKVKSKDVRLTGNWTKDDGW

SEQ ID NO: 59 - protein, 194 aa, Humicolopsis cephalosporioides
APTPAPVELERRTPPNIPTTASAKSLLAGLTVAAQGPQTGYSRDLFPHWITISGSCNTRETVLKRDGTGVVTDSACASTAGSWYSPYDGATWTAASDVDIDHMVPLSNAWKSGAAQWTTARRQDFANDLTNPQLFAVTDNVNQEKGDKGPEDWKPSLTSYYCTYAKAWVKVKSVWALTITSAEKSALTTMLNTC

SEQ ID NO: 60 - protein, 190 aa, Neosartorya massa
IPAPVALPTPPGIPSAATAESELAALTVAAQGSSSGYSRDLFPHWISQGGSCNTREVVLARDGSGVVKDSNCYPTSGSWYSPYDGATWTQASDVDIDHVVPLANAWRSGASKWTTSQRQAFANDLTNPQLMAVTDNVNQAKGDDGPEAWKPPLTSYYCTYAKMWVRVKYVYDLTITSAEKSALVSMLDTC

SEQ ID NO: 61 - protein, 191 aa, Roussoella intermedia
APTPALLPRAPPNIPSTATAKSQLAALTVAAQGPQDGYSRDLFPHWITQSGSCNTREVVLKRDGTNVVQDSSCAATSGTWVSPFDGATWTAASDVDIDHLVPLSNAWKSGAASWTTARRQSFANDLTNPQLLAVTDEVNQAKGDKGPEAWKPPLASYHCTYAKMWVKVKSTYSLTITSAEKSALTTMLNTC

SEQ ID NO: 62 - protein, 191 aa, Pleosporales
LPTPSLVKRTPPNIPSTTSAKSLLAGLTVAAQGPQDGYSRDLFPHWITISGTCNTRETVLKRDGTNVVTDSACASTSGSWYSTYDGATWTAASDVDIDHVVPLSNAWKSGAASWTTARRQSFANDLTNPQLIAVTDSVNQSKGDKGPESWKPPLTSYHCTYAKMWVKVKDVYSLTVTSAEKSALTTMLNTC

SEQ ID NO: 63 - protein, 192 aa, Phaeosphaeria sp.
LPAPIHLTARAPPNIPSASEARTQLAGLTVAAQGPQDGYSRDLFPHWITQSGTCNTRETVLKRDGTNVVTNSACASTSGSWFSPYDGATWTAASDVDIDHMVPLSNAWKSGAASWTTARRQAFANDLTNPQLLAVTDNVNQAKGDKGPEDWKPPLTSYYCTYARMWVKVKSVYALTVTSAEKSALTSMLGTC

SEQ ID NO: 64 - protein, 189 aa, Didymosphaeria futilis
LPTPNTLEARAPPNIPSTSAAQSQLSALTVAAQGPQTGYSRDLFPHWITQSGTCNTRETVLKRDGTNVLTDSACASTSGSWKSPYDGATWTAASDVDIDHVVPLSNAWKSGAASWTTARRQSFANDLTNPQLIAVTDNVNQAKGDKGPEDWKPPLTSYYCTYAKMWVKVKSVYSLTITSAEKSALTMLA

SEQ ID NO: 65 - protein, 109 aa, Bacillus licheniformis
ARYDDILYFPASRYPETGAHISDAIKAGHSDVCTIERSGADKRRQESLKGIPTKPGFDRDEWPMAMCEEGGKGASVRYVSSSDNRGAGSWVGNRLSGFADGTRILFIVQ

SEQ ID NO: 66 - protein, 110 aa, Bacillus subtilis
ASSYDKVLYFPLSRYPETGSHIRDAIAEGHPDICTIDRDGADKRREESLKGIPTKPGYDRDEWPMAVCEEGGAGADVRYVTPSDNRGAGSWVGNQMSSYPDGTRVLFIVQ

SEQ ID NO: 67 - protein, 221 aa, Aspergillus oryzae
VPVNPEPDATSVENVALKTGSGDSQSDPIKADLEVKGQSALPFDVDCWAILCKGAPNVLQRVNEKTKNSNRDRSGANKGPFKDPQKWGIKALPPKNPSWSAQDFKSPEEYAFASSLQGGTNAILAPVNLASQNSQGGVLNGFYSANKVAQFDPSKPQQTKGTWFQITKFTGAAGPYCKALGSNDKSVCDKNKNIAGDWGFDPAKWAYQYDEKNNKFNYVGK

SEQ ID NO: 68 - protein, 188 aa, Trichoderma harzianum
APAPMPTPPGIPTESSARTQLAGLTVAVAGSGTGYSRDLFPTWDAISGNCNAREYVLKRDGEGVQVNNACESQSGTWISPYDNASFTNASSLDIDHMVPLKNAWISGASSWTTAQREALANDVSRPQLWAVSASANRSKGDRSPDQWKPPLTSFYCTYAKSWIDVKSFYKLTITSAEKTALSSMLDTC

SEQ ID NO: 69 - protein, 5 aa, Artificial
  Motif
  MISC_FEATURE (1)..(1): Xaa = Thr (T) or Asp (D) or Ser (S)
  MISC_FEATURE (2)..(2): Xaa = Gly (G) or Asn (N)
XXPQL

SEQ ID NO: 70 - protein, 5 aa, Artificial
  Motif
  MISC_FEATURE (1)..(1): Xaa = F (phe) or L (Leu) or Y (Tyr) or I (Ile)
  MISC_FEATURE (3)..(3): Xaa = N (Asn) or R (Arg)
  MISC_FEATURE (5)..(5): Xaa = L (Leu) or I (Ile) or P (Phe) or V (Val)
XAXDX

SEQ ID NO: 71 - protein, 4 aa, Artificial
  Motif
  MISC_FEATURE (2)..(2): Xaa= Asp (D) or Asn (N)
  MISC_FEATURE (4)..(4): Xaa= Ala (A) or Arg (R)
CXTX

SEQ ID NO: 72 - protein, 4 aa, Artificial
  Motif
  MISC_FEATURE (1)..(1): Xaa = Asp (D) or Gln (Q)
  MISC_FEATURE (2)..(2): Xaa = Ile (I) or Val (V)
XXDH

SEQ ID NO: 73 - protein, 7 aa, Artificial
  Motif
  MISC_FEATURE (1)..(1): Xaa = Asp (D) or Met (M) or Leu (L)
  MISC_FEATURE (2)..(2): Xaa = Ser (S) or Thr (T)
  MISC_FEATURE (7)..(7): Xaa = Asp (D) or Asn (N)
XXGYSRX

SEQ ID NO: 74 - protein, 8 aa, Artificial
  Motif
  MISC_FEATURE (3)..(3): Xaa = any amino acid
ASXNRSKG

SEQ ID NO: 75 - protein, 8 aa, Artificial
  Motif
  MISC_FEATURE (1)..(1): Xaa = Val (V) or Ile (I)
  MISC_FEATURE (4)..(4): Xaa = Ser (S) or Ala (A)
XPLXNAWK

SEQ ID NO: 76 - protein, 4 aa, Artificial
  Motif
NPQL

SEQ ID NO: 77 - protein, 4 aa, Artificial
  Motif
  MISC_FEATURE (2)..(2): Xaa = Gln (Q) or Glu(E)
  MISC_FEATURE (4)..(4): Xaa = Trp (W) or Tyr (Y)
PXLX

SEQ ID NO: 78 - protein, 4 aa, Artificial
  Motif
  MISC_FEATURE (1)..(1): Xaa=Lys (K) or His (H) or Glu (E)
XNAW

SEQ ID NO: 79 - protein, 269 aa, Bacillus lentus
AQSVPWGISRVQAPAAHNRGLTGSGVKVAVLDTGISTHPDLNIRGGASFVPGEPSTQDGNGHGTHVAGTIAALNNSIGVLGVAPSAELYAVKVLGASGSGSVSSIAQGLEWAGNNGMHVANLSLGSPSPSATLEQAVNSATSRGVLVVAASGNSGAGSISYPARYANAMAVGATDQNNNRASFSQYGAGLDIVAPGVNVQSTYPGSTYASLNGTSMATPHVAGAAALVKQKNPSWSNVQIRNHLKNTATSLGSTNLYGSGLVNAEAATR

SEQ ID NO: 80 - protein, 275 aa, Bacillus amyloliquefaciens [sequence omitted]

SEQ ID NO: 81 - protein, 311 aa, Bacillus subtilis [sequence omitted]

SEQ ID NO: 82 - protein, 4 aa, Artificial
  Motif
EYTV

SEQ ID NO: 83 - protein, 4 aa, Artificial
  Motif
  MISC_FEATURE (1)..(1): Xaa=Y (Tyr) or R (Arg) or F (Phe)
  MISC_FEATURE (3)..(3): Xaa=A (Ala) or Y (Tyr) or F (Phe) or W (Trp) or C (Cys)
XEXD

SEQ ID NO: 84 - protein, 4 aa, Artificial
  Motif
IGGD

SEQ ID NO: 85 - protein, 4 aa, Artificial
  Motif
HTGA

SEQ ID NO: 86 - protein, 144 aa, Paenibacillus sp-18057
GCGQIGVDSPQGIASHSAEAPGTQDVSRQAPLTGFKEVADYIRSYGALPDNFITKKEAERLGWVPSEGNLGKVAPGKSIGGDRFGNREGLLPKEKNRIWYEADINYEGGTRGADRIVFSNDGLIYMTTDHYRSFTDITEGGPDP

SEQ ID NO: 87 - protein, 119 aa, Paenibacillus sp-62770
LTVDDSTQTQAVLNQFDEVANYLAEHQELPDNYITKKEARALGWEPSEGNLQDVAPGKSIGGDIFQNREGLLPKKKGRTWYEADINYSGGTRGSDRILYSSDGLIYKTTDHYRTFEQIK

SEQ ID NO: 88 - protein, 134 aa, Amycolatopsis azurea
FVKDGISGDDTKSSSAPASSSAQPKPSGAAKGKVAGEESGLPVKPLTGLPSQASDTWKLITAGGPYPYPRNDDVTFQNREKVLPAKDSGYYREYTVKTPGSPDRGARRLVTGTGKELYYTEDHYKSFVVVDPSR

SEQ ID NO: 89 - protein, 158 aa, Enviromental sample E
CSILDINYDGPEMPKLEEPSEGEIPNDEIPDIEIPEDEIPEGESLIIEDGQYTRKDEVAEYIHIFGRLPENYITKNEAMDLGWDASSGNLWDVTDEMSIGGDRFGNREGLLPEASGRKWYEADIDYEGGRRNAKRIVFSDDGLIYYTDDHYASFEKLY

SEQ ID NO: 90 - protein, 114 aa, Acremonium alcalophilum
APSGQLEKRATTCGSTYYSTSQVSAAASAACNHVRAGTRAGSSTYPHAYNNYEGFNFPISGPYQLFPLRTSGVYTGGAPGPDRVIINRNTCAIAGQITHTGAPGNAFVGCSGTY

SEQ ID NO: 91 - protein, 157 aa, Bacillus amyloliquefaciens
MMKMEGIALKKRLSWISVCLLVLVSAAGMLFSTAAKTETSSHKAHTEAQVINTFDGVADYLQTYHKLPDNYITKSEAQALGWVASKGNLADVAPGKSIGGDIFSNREGKLPGKSGRTWREADINYTSGFRNSDRILYSSDWLIYKTTDHYQTFTKIR

SEQ ID NO: 92 - protein, 139 aa, Stenotrophomonas rhizophila
IKEAQRAPAPQFAPSLTQPGADPAPIDNAPTHPGATATRTHDALPAFLPAEARQTLILIQRGGPYPHRQDGGVFSNREQRLPDRPRGYYREYTVDTPGAGNRGARRIVTGGTPPTGWFYTDDHYETFRSFEVPPAGSWQ

SEQ ID NO: 93 - protein, 136 aa, Erwinia persicina
REHGQSEKPAVRPSASVSAPQHDSNDIDVLTQQQRVADYLRQHQQLPGYYIRKGEARQQGWDPSKGNLCQVLPGRAIGGDRFSNREGGLPQKNGRRWFEADVNYACGRRGTDRLLYSSDGLIYLTRDHYRHFQQVN

SEQ ID NO: 94 - protein, 119 aa, Paenibacillus tundrae
VSLNGSSQEKATLTQFDEVAKYISEHNELPENYITKKEARELGWEPSKGNLEKVAPGKSIGGDVFQNREGLLPKKKGRTWYEADINYSGGTRGSDRILYSNDGLIYKTTDHYRTFEQIE

SEQ ID NO: 95 - protein, 117 aa, Saccharothrix sp-62935
LTGTSSDPAPPSASATVPGADSGLPVEPLSSLPAQVKTTWELIGRGGPFPHPRNDGVTFQNREKLLPAKPSDYYREYTVPTPGSDDRGARRLVTGSSDEVYYTADHYESFVVVDVTG

SEQ ID NO: 96 - protein, 108 aa, Saccharopolyspora endophytica
DSPSTEVPGASQSGLQVQQLSKLPPETGKTYQLIVKGGPFPYPGKDGSVFGNREGELPEQKSGYYHEYTVPTPGSKDRGARRLVTGGQDEVYYTGDHYESFVVVDTAG

SEQ ID NO: 97 - protein, 120 aa, Amycolatopsis circi
SDSPAPSSSSGAPAAASGKVPGADSKLPVKPLSSLPSQAKDTWSLIHKGGPYPYPRNDDVVFQNREKKLPAEKNGYYHEYTVKTPGSPDRGARRLITGAGKELYYTGDHYASFVVVDPAR

SEQ ID NO: 98 - protein, 119 aa, Paenibacillus sp-62770
LSVGDTNQTHAVLNQFDEVANYLAEHQELPDNYITKKEARALGWEPSEGNLQDMAPGKSIGGDIFQNREGLLPKKKGRTWYEADINYSGGTRGSDRILYSSDGLIYKTTDHYRTFEQIK

SEQ ID NO: 99 - protein, 117 aa, Paenibacillus sp-18006
LDQTTTTASQDMGFDEVAKYISEHNALPPNYITKKEARALGWEPSEGNLQEVAPGKSIGGDVFRNREGLLPNKKGRTWYEADIHYAGGRRGSDRILYSNDGLIYKTTDHYESFEQLK

SEQ ID NO: 100 - protein, 156 aa, Paenibacillus sp-62724
TENQSPAFQEPNSSVSNSSPTEQPQPSPIPTNSEVGENVQAPLTSFKAVSDYIREHHTLPANFITKKEAEQLGWVPAKGNLDQVAPGKSIGGDRFGNREGLLPKAKNRIWYEADINYTKKSRGADRVLYSNDGLIYMTTDHYKSFTDITKEGSVPE

SEQ ID NO: 101 - protein, 115 aa, Alkalimonas sp-62516
QPSVTPGAEVTQSGSGAQPRMSAQQLELQKTLQRIQGNGPFPYDRDGITFHNRERLLPIKPRGYYREYTVDTPGLSHRGPRRVVTGGNPPVVFYYTEDHYQSFRRISGDPYERIH

SEQ ID NO: 102 - protein, 108 aa, Nonomuraea dietziae
ALPEESRAAPPPAALPEKALSALPPEAAKTWRLIQSDGPFPYRRDGVVFQNRERILPQQKRGYYHEYTVPTPGSRDRGARRLVTGTGVDELYYTGDHYRSFVAVDVKR

SEQ ID NO: 103 - protein, 116 aa, Trichoderma harzianum
APLDELTKRDTATCGKVFYSASAVSAASNAACNYVRAGSTAGGSTYPHVYNNYEGFRFKGLSKPFYEFPILSSGKTYTGGSPGADRVVINGQCSIAGIITHTGASGNAFVACAGTS

SEQ ID NO: 104 - protein, 112 aa, Fusarium solani
GPIESRQSATTCGNTAYSAAQVRAAANAACSYYRADDTAGSSTYPHTFNNREGFDFLVSGPYQEFPIRSSGVYTGGSPGADRVVINTSCQYAGAITHTGASGNNFVGCSGTN